European Patent Specification EP 2 885 416 B1, published January 3, 2024. Title: Large Scale Enzymatic Synthesis of Oligosaccharides. Applicant: Academia Sinica Wong, Chi-Huey Tsai, Tsung-I Wu, Chung-Yi. Application N/A. The sequence listing filed with the application follows.

SEQUENCE LISTING (30 sequences)

SEQ ID NO: 1 - DNA, 46 bp, Artificial Sequence
  Synthetic oligonucleotide
ctgtattttcagggagcgatcgctatgagtctgaaagaaaaaacab

SEQ ID NO: 2 - DNA, 44 bp, Artificial Sequence
  Synthetic oligonucleotide
gcctcgagtcattacgtttaaactcagcactgtcctgctccttg

SEQ ID NO: 3 - DNA, 44 bp, Artificial Sequence
  Synthetic oligonucleotide
ctgtattttcagggagcgatcgctatggcttctacggttgattc

SEQ ID NO: 4 - DNA, 46 bp, Artificial Sequence
  Synthetic oligonucleotide
gcctcgagtcattacgtttaaactcaatcttcaacagaaaatttgc

SEQ ID NO: 5 - DNA, 35 bp, Artificial Sequence
  Synthetic oligonucleotide
gatataccatggaaatggacatcgttttcgcggcg

SEQ ID NO: 6 - DNA, 33 bp, Artificial Sequence
  Synthetic oligonucleotide
gtggtgctcgaggtagattttacgcaggaaacg

SEQ ID NO: 7 - DNA, 50 bp, Artificial Sequence
  Synthetic oligonucleotide
ctgtattttcagggagcgatcgctatgaacaagacttatgattttaaaag

SEQ ID NO: 8 - DNA, 48 bp, Artificial Sequence
  Synthetic oligonucleotide
gcctcgagtcattacgtttaaacttaaatgtatgaatatactatcttc

SEQ ID NO: 9 - DNA, 45 bp, Artificial Sequence
  Synthetic oligonucleotide
ctgtattttcagggagcgatcgctatgttgaataatgctatgagc

SEQ ID NO: 10 - DNA, 44 bp, Artificial Sequence
  Synthetic oligonucleotide
gcctcgagtcattacgtttaaactcactttttctttaccggacg

SEQ ID NO: 11 - DNA, 32 bp, Artificial Sequence
  Synthetic oligonucleotide
gatataccatggaaaactgcccgctggtttct

SEQ ID NO: 12 - DNA, 34 bp, Artificial Sequence
  Synthetic oligonucleotide
gtggtgctcgaggaagataacgttgattttacgg

SEQ ID NO: 13 - DNA, 36 bp, Artificial Sequence
  Synthetic oligonucleotide
cagggagcgatcgctatgcaaaaactactatcttta

SEQ ID NO: 14 - DNA, 35 bp, Artificial Sequence
  Synthetic oligonucleotide
cattacgtttaaacttatgatcgtgatacttggaa

SEQ ID NO: 15 - DNA, 45 bp, Artificial Sequence
  Synthetic oligonucleotide
ctgtattttcagggagcgatcgctatggcgttcaaagttgttcag

SEQ ID NO: 16 - DNA, 45 bp, Artificial Sequence
  Synthetic oligonucleotide
gcctcgagtcattacgtttaaacttacgcgttgtatttctgagat

SEQ ID NO: 17 - DNA, 36 bp, Artificial Sequence
  Synthetic oligonucleotide
cagggagcgatcgctatgacggcaattgccccggtt

SEQ ID NO: 18 - DNA, 35 bp, Artificial Sequence
  Synthetic oligonucleotide
cattacgtttaaacttatgcgagagccaatttctg

SEQ ID NO: 19 - DNA, 36 bp, Artificial Sequence
  Synthetic oligonucleotide
gatataccatggaaacaaatattgcgatcattcctg

SEQ ID NO: 20 - DNA, 36 bp, Artificial Sequence
  Synthetic oligonucleotide
gtggtgctcgagtttattggataaaatttccgcgag

SEQ ID NO: 21 - DNA, 35 bp, Artificial Sequence
  Synthetic oligonucleotide
gatataccatggaaatgaacaacgacaactctacc

SEQ ID NO: 22 - DNA, 34 bp, Artificial Sequence
  Synthetic oligonucleotide
gtggtgctcgaggatgtcagagatcagtttgatg

SEQ ID NO: 23 - DNA, 47 bp, Artificial Sequence
  Synthetic oligonucleotide
ctgtattttcagggagcgatcgctatgaaaaagaccaaaattgtttg

SEQ ID NO: 24 - DNA, 43 bp, Artificial Sequence
  Synthetic oligonucleotide
gcctcgagtcattacgtttaaacttacaggacgtgaacagatg

SEQ ID NO: 25 - DNA, 36 bp, Artificial Sequence
  Synthetic oligonucleotide
cagggagcgatcgctatgagcttactcaacgtccct

SEQ ID NO: 26 - DNA, 35 bp, Artificial Sequence
  Synthetic oligonucleotide
cattacgtttaaacttatttattctttgcgcgctc

SEQ ID NO: 27 - DNA, 936 bp, Escherichia coli
atggacatcgttttcgcggcggacgacaactacgcggcgtacctgtgcgttgcggcgaaatctgttgaagcggcgcacccggacaccgaaatccgtttccacgttctggacgcgggtatctctgaagcgaaccgtgcggcggttgcggcgaacctgcgtggtggtggtggtaacatccgtttcatcgacgttaacccggaagacttcgcgggtttcccgctgaacatccgtcacatctctatcaccacctacgcgcgtctgaaactgggtgaatacatcgcggactgcgacaaagttctgtacctggacatcgacgttctggttcgtgactctctgaccccgctgtgggacaccgacctgggtgacaactggctgggtgcgtgcatcgacctgttcgttgaacgtcaggaaggttacaaacagaaaatcggtatggcggacggtgaatactacttcaacgcgggtgttctgctgatcaacctgaaaaaatggcgtcgtcacgacatcttcaaaatgtcttgcgaatgggttgaacagtacaaagacgttatgcagtaccaggaccaggacatcctgaacggtctgttcaaaggtggtgtttgctacgcgaactctcgtttcaacttcatgccgaccaactacgcgttcatggcgaaccgtttcgcgtctcgtcacaccgacccgctgtaccgtgaccgtaccaacaccgttatgccggttgcggtttctcactactgcggtccggcgaaaccgtggcaccgtgactgcaccgcgtggggtgcggaacgtttcaccgaactggcgggttctctgaccaccgttccggaagaatggcgtggtaaactggcggttccgcaccgtatgttctctaccaaacgtatgctgcagcgttggcgtcgtaaactgtctgcgcgtttcctgcgtaaaatctactga

SEQ ID NO: 28 - DNA, 972 bp, Escherichia coli
atggaaaactgcccgctggtttctgttatcgtttgcgcgtacaacgcggaacagtacatcgacgaatctatctcttctatcatcaaccagacctacgaaaacctggaaatcatcgttatcaacgacggttctaccgacctgaccctgtctcacctggaagaaatctctaaactggacaaacgtatcaaaatcatctctaacaaatacaacctgggtttcatcaactctctgaacatcggtctgggttgcttctctggtaaatacttcgcgcgtatggacgcggacgacatcgcgaaaccgtcttggatcgaaaaaatcgttacctacctggaaaaaaacgaccacatcaccgcgatgggttcttacctggaaatcatcgttgaaaaagaatgcggtatcatcggttctcagtacaaaaccggtgacatctggaaaaacccgctgctgcacaacgacatctgcgaagcgatgctgttctacaacccgatccacaacaacaccatgatcatgcgtgcgaacgtttaccgtgaacacaaactgatcttcaacaaagactacccgtacgcggaagactacaaattctggtctgaagtttctcgtctgggttgcctggcgaactacccggaagcgctggttaaataccgtctgcacggtaaccagacctcttctgtttacaaccacgaacagaacgaaaccgcgaaaaaaatcaaacgtgaaaacatcacctactacctgaacaaaatcggtatcgacatcaaagttatcaactctgtttctctgctggaaatctaccacgttgacaaatctaacaaagttctgaaatctatcctgtacgaaatgtacatgtctctggacaaatacaccatcacctctctgctgcacttcatcaaataccacctggaactgttcgacctgaaacagaacctgaaaatcatcaaaaaattcatccgtaaaatcaacgttatcttctag

SEQ ID NO: 29 - DNA, 903 bp, Escherichia coli
atggcgttcaaagttgttcagatctgcggtggtctgggtaaccagatgttccagtacgcgttcgcgaaatctctgcagaaacactctaacaccccggttctgctggacatcacctctttcgactggtctgaccgtaaaatgcagctggaactgttcccgatcgacctgccgtacgcgtctgcgaaagaaatcgcgatcgcgaaaatgcagcacctgccgaaactggttcgtgacgcgctgaaatgcatgggtttcgaccgtgtttctcaggaaatcgttttcgaatacgaaccgaaactgctgaaaccgtctcgtctgacctacttcttcggttacttccaggacccgcgttacttcgacgcgatctctccgctgatcaaacagaccttcaccctgccgccgccgccggaaaacaacaaaaacaacaacaaaaaagaagaagaataccagtgcaaactgtctctgatcctggcggcgaaaaactctgttttcgttcacatccgtcgtggtgactacgttggtatcggttgccagctgggtatcgactaccagaaaaaagcgctggaatacatggcgaaacgtgttccgaacatggaactgttcgttttctgcgaagacctggaattcacccagaacctggacctgggttacccgttcatggacatgaccacccgtgacaaagaagaagaagcgtactgggacatgctgctgatgcagtcttgccagcacggtatcatcgcgaactctacctactcttggtgggcggcgtacctgatcgaaaacccggaaaaaatcatcatcggtccgaaacactggctgttcggtcacgaaaacatcctgtgcaaagaatgggttaaaatcgaatctcacttcgaagttaaatctcagaaatacaacgcgtaa

SEQ ID NO: 30 - DNA, 1146 bp, Escherichia coli
atgaacaacgacaactctaccaccaccaacaacaacgcgatcgaaatctacgttgaccgtgcgaccctgccgaccatccagcagatgaccaaaatcgtttctcagaaaacctctaacaaaaaactgatctcttggtctcgttacccgatcaccgacaaatctctgctgaaaaaaatcaacgcggaattcttcaaagaacagttcgaactgaccgaatctctgaaaaacatcatcctgtctgaaaacatcgacaacctgatcatccacggtaacaccctgtggtctatcgacgttgttgacatcatcaaagaagttaacctgctgggtaaaaacatcccgatcgaactgcacttctacgacgacggttctgcggaatacgttcgtatctacgaattctctaaactgccggaatctgaacagaaatacaaaacctctctgtctaaaaacaacatcaaattctctatcgacggtaccgactctttcaaaaacaccatcgaaaacatctacggtttctctcagctgtacccgaccacctaccacatgctgcgtgcggacatcttcgacaccaccctgaaaatcaacccgctgcgtgaactgctgtctaacaacatcaaacagatgaaatgggactacttcaaagacttcaactacaaacagaaagacatcttctactctctgaccaacttcaacccgaaagaaatccaggaagacttcaacaaaaactctaacaaaaacttcatcttcatcggttctaactctgcgaccgcgaccgcggaagaacagatcaacatcatctctgaagcgaaaaaagaaaactcttctatcatcaccaactctatctctgactacgacctgttcttcaaaggtcacccgtctgcgaccttcaacgaacagatcatcaacgcgcacgacatgatcgaaatcaacaacaaaatcccgttcgaagcgctgatcatgaccggtatcctgccggacgcggttggtggtatgggttcttctgttttcttctctatcccgaaagaagttaaaaacaaattcgttttctacaaatctggtaccgacatcgaaaacaactctctgatccaggttatgctgaaactgaacctgatcaaccgtgacaacatcaaactgatctctgacatctaa